European Patent Application EP 4 144 377 A1, published March 8, 2023. Title: ANTIBODY-DRUG CONJUGATE COMPRISING MODIFIED ANTIBODY. Applicant: ALTEOGEN, INC. Application EP. The sequence listing filed with the application follows.

SEQUENCE LISTING (128 sequences)

SEQ ID NO: 1 - protein, 5 aa, synthetic construct
  REGION 1..5: note = Motif
ACGHA

SEQ ID NO: 2 - protein, 5 aa, synthetic construct
  REGION 1..5: note = Motif
AHGCA

SEQ ID NO: 3 - protein, 5 aa, synthetic construct
  REGION 1..5: note = Motif
  SITE 2: note = MISC_FEATURE - Xaa is any amino acid residue
AXGHA

SEQ ID NO: 4 - protein, 5 aa, synthetic construct
  REGION 1..5: note = Motif
  SITE 4: note = MISC_FEATURE - Xaa is any amino acid residue
AHGXA

SEQ ID NO: 5 - protein, 10 aa, synthetic construct
  REGION 1..10: note = Motif
ACGHAACGHA

SEQ ID NO: 6 - protein, 10 aa, synthetic construct
  REGION 1..10: note = Motif
ACGHAAHGCA

SEQ ID NO: 7 - protein, 10 aa, synthetic construct
  REGION 1..10: note = Motif
  SITE 7: note = MISC_FEATURE - Xaa is any amino acid residue
ACGHAAXGHA

SEQ ID NO: 8 - protein, 10 aa, synthetic construct
  REGION 1..10: note = Motif
  SITE 9: note = MISC_FEATURE - Xaa is any amino acid residue
ACGHAAHGXA

SEQ ID NO: 9 - protein, 10 aa, synthetic construct
  REGION 1..10: note = Motif
AHGCAAHGCA

SEQ ID NO: 10 - protein, 10 aa, synthetic construct
  REGION 1..10: note = Motif
AHGCAACGHA

SEQ ID NO: 11 - protein, 10 aa, synthetic construct
  REGION 1..10: note = Motif
  SITE 7: note = MISC_FEATURE - Xaa is any amino acid residue
AHGCAAXGHA

SEQ ID NO: 12 - protein, 10 aa, synthetic construct
  REGION 1..10: note = Motif
  SITE 9: note = MISC_FEATURE - Xaa is any amino acid residue
AHGCAAHGXA

SEQ ID NO: 13 - protein, 10 aa, synthetic construct
  REGION 1..10: note = Motif
  SITE 2: note = MISC_FEATURE - Xaa is any amino acid residue
  SITE 7: note = MISC_FEATURE - Xaa is any amino acid residue
AXGHAAXGHA

SEQ ID NO: 14 - protein, 10 aa, synthetic construct
  REGION 1..10: note = Motif
  SITE 2: note = MISC_FEATURE - Xaa is any amino acid residue
AXGHAACGHA

SEQ ID NO: 15 - protein, 10 aa, synthetic construct
  REGION 1..10: note = Motif
  SITE 2: note = MISC_FEATURE - Xaa is any amino acid residue
AXGHAAHGCA

SEQ ID NO: 16 - protein, 10 aa, synthetic construct
  REGION 1..10: note = Motif
  SITE 2: note = MISC_FEATURE - Xaa is any amino acid residue
  SITE 9: note = MISC_FEATURE - Xaa is any amino acid residue
AXGHAAHGXA

SEQ ID NO: 17 - protein, 10 aa, synthetic construct
  REGION 1..10: note = Motif
  SITE 4: note = MISC_FEATURE - Xaa is any amino acid residue
  SITE 9: note = MISC_FEATURE - Xaa is any amino acid residue
AHGXAAHGXA

SEQ ID NO: 18 - protein, 10 aa, synthetic construct
  REGION 1..10: note = Motif
  SITE 4: note = MISC_FEATURE - Xaa is any amino acid residue
AHGXAACGHA

SEQ ID NO: 19 - protein, 10 aa, synthetic construct
  REGION 1..10: note = Motif
  SITE 4: note = MISC_FEATURE - Xaa is any amino acid residue
AHGXAAHGCA

SEQ ID NO: 20 - protein, 10 aa, synthetic construct
  REGION 1..10: note = Motif
  SITE 4: note = MISC_FEATURE - Xaa is any amino acid residue
  SITE 7: note = MISC_FEATURE - Xaa is any amino acid residue
AHGXAAXGHA

SEQ ID NO: 21 - protein, 10 aa, synthetic construct
  REGION 1..10: note = Motif
ACGHAASGHA

SEQ ID NO: 22 - protein, 10 aa, synthetic construct
  REGION 1..10: note = Motif
ACGHAAHGSA

SEQ ID NO: 23 - protein, 10 aa, synthetic construct
  REGION 1..10: note = Motif
AHGCAASGHA

SEQ ID NO: 24 - protein, 10 aa, synthetic construct
  REGION 1..10: note = Motif
AHGCAAHGSA

SEQ ID NO: 25 - protein, 10 aa, synthetic construct
  REGION 1..10: note = Motif
ASGHAASGHA

SEQ ID NO: 26 - protein, 10 aa, synthetic construct
  REGION 1..10: note = Motif
ASGHAACGHA

SEQ ID NO: 27 - protein, 10 aa, synthetic construct
  REGION 1..10: note = Motif
ASGHAAHGCA

SEQ ID NO: 28 - protein, 10 aa, synthetic construct
  REGION 1..10: note = Motif
ASGHAAHGSA

SEQ ID NO: 29 - protein, 10 aa, synthetic construct
  REGION 1..10: note = Motif
AHGSAAHGSA

SEQ ID NO: 30 - protein, 10 aa, synthetic construct
  REGION 1..10: note = Motif
AHGSAACGHA

SEQ ID NO: 31 - protein, 10 aa, synthetic construct
  REGION 1..10: note = Motif
AHGSAAHGCA

SEQ ID NO: 32 - protein, 10 aa, synthetic construct
  REGION 1..10: note = Motif
AHGSAASGHA

SEQ ID NO: 33 - protein, 10 aa, synthetic construct
  REGION 1..10: note = Motif
ACGHAAAGHA

SEQ ID NO: 34 - protein, 10 aa, synthetic construct
  REGION 1..10: note = Motif
ACGHAAHGAA

SEQ ID NO: 35 - protein, 10 aa, synthetic construct
  REGION 1..10: note = Motif
AHGCAAAGHA

SEQ ID NO: 36 - protein, 10 aa, synthetic construct
  REGION 1..10: note = Motif
AHGCAAHGAA

SEQ ID NO: 37 - protein, 10 aa, synthetic construct
  REGION 1..10: note = Motif
AAGHAAAGHA

SEQ ID NO: 38 - protein, 10 aa, synthetic construct
  REGION 1..10: note = Motif
AAGHAACGHA

SEQ ID NO: 39 - protein, 10 aa, synthetic construct
  REGION 1..10: note = Motif
AAGHAAHGCA

SEQ ID NO: 40 - protein, 10 aa, synthetic construct
  REGION 1..10: note = Motif
AAGHAAHGAA

SEQ ID NO: 41 - protein, 10 aa, synthetic construct
  REGION 1..10: note = Motif
AHGAAAHGAA

SEQ ID NO: 42 - protein, 10 aa, synthetic construct
  REGION 1..10: note = Motif
AHGAAACGHA

SEQ ID NO: 43 - protein, 10 aa, synthetic construct
  REGION 1..10: note = Motif
AHGAAAHGCA

SEQ ID NO: 44 - protein, 10 aa, synthetic construct
  REGION 1..10: note = Motif
AHGAAAAGHA

SEQ ID NO: 45 - protein, 10 aa, synthetic construct
  REGION 1..10: note = Motif
ACGHAATGHA

SEQ ID NO: 46 - protein, 10 aa, synthetic construct
  REGION 1..10: note = Motif
ACGHAAHGTA

SEQ ID NO: 47 - protein, 10 aa, synthetic construct
  REGION 1..10: note = Motif
AHGCAATGHA

SEQ ID NO: 48 - protein, 10 aa, synthetic construct
  REGION 1..10: note = Motif
AHGCAAHGTA

SEQ ID NO: 49 - protein, 10 aa, synthetic construct
  REGION 1..10: note = Motif
ATGHAATGHA

SEQ ID NO: 50 - protein, 10 aa, synthetic construct
  REGION 1..10: note = Motif
ATGHAACGHA

SEQ ID NO: 51 - protein, 10 aa, synthetic construct
  REGION 1..10: note = Motif
ATGHAAHGCA

SEQ ID NO: 52 - protein, 10 aa, synthetic construct
  REGION 1..10: note = Motif
ATGHAAHGTA

SEQ ID NO: 53 - protein, 10 aa, synthetic construct
  REGION 1..10: note = Motif
AHGTAAHGTA

SEQ ID NO: 54 - protein, 10 aa, synthetic construct
  REGION 1..10: note = Motif
AHGTAACGHA

SEQ ID NO: 55 - protein, 10 aa, synthetic construct
  REGION 1..10: note = Motif
AHGTAAHGCA

SEQ ID NO: 56 - protein, 10 aa, synthetic construct
  REGION 1..10: note = Motif
AHGTAATGHA

SEQ ID NO: 57 - protein, 10 aa, synthetic construct
  REGION 1..10: note = Motif
ACGHAAYGHA

SEQ ID NO: 58 - protein, 10 aa, synthetic construct
  REGION 1..10: note = Motif
ACGHAAHGYA

SEQ ID NO: 59 - protein, 10 aa, synthetic construct
  REGION 1..10: note = Motif
AHGCAAYGHA

SEQ ID NO: 60 - protein, 10 aa, synthetic construct
  REGION 1..10: note = Motif
AHGCAAHGYA

SEQ ID NO: 61 - protein, 10 aa, synthetic construct
  REGION 1..10: note = Motif
AYGHAAYGHA

SEQ ID NO: 62 - protein, 10 aa, synthetic construct
  REGION 1..10: note = Motif
AYGHAACGHA

SEQ ID NO: 63 - protein, 10 aa, synthetic construct
  REGION 1..10: note = Motif
AYGHAAHGCA

SEQ ID NO: 64 - protein, 10 aa, synthetic construct
  REGION 1..10: note = Motif
AYGHAAHGYA

SEQ ID NO: 65 - protein, 10 aa, synthetic construct
  REGION 1..10: note = Motif
AHGYAAHGYA

SEQ ID NO: 66 - protein, 10 aa, synthetic construct
  REGION 1..10: note = Motif
AHGYAACGHA

SEQ ID NO: 67 - protein, 10 aa, synthetic construct
  REGION 1..10: note = Motif
AHGYAAHGCA

SEQ ID NO: 68 - protein, 10 aa, synthetic construct
  REGION 1..10: note = Motif
AHGYAAYGHA

SEQ ID NO: 69 - protein, 10 aa, synthetic construct
  REGION 1..10: note = Motif
ACGHAADGHA

SEQ ID NO: 70 - protein, 10 aa, synthetic construct
  REGION 1..10: note = Motif
ACGHAAHGDA

SEQ ID NO: 71 - protein, 10 aa, synthetic construct
  REGION 1..10: note = Motif
AHGCAADGHA

SEQ ID NO: 72 - protein, 10 aa, synthetic construct
  REGION 1..10: note = Motif
AHGCAAHGDA

SEQ ID NO: 73 - protein, 10 aa, synthetic construct
  REGION 1..10: note = Motif
ADGHAADGHA

SEQ ID NO: 74 - protein, 10 aa, synthetic construct
  REGION 1..10: note = Motif
ADGHAACGHA

SEQ ID NO: 75 - protein, 10 aa, synthetic construct
  REGION 1..10: note = Motif
ADGHAAHGCA

SEQ ID NO: 76 - protein, 10 aa, synthetic construct
  REGION 1..10: note = Motif
ADGHAAHGDA

SEQ ID NO: 77 - protein, 10 aa, synthetic construct
  REGION 1..10: note = Motif
AHGDAAHGDA

SEQ ID NO: 78 - protein, 10 aa, synthetic construct
  REGION 1..10: note = Motif
AHGDAACGHA

SEQ ID NO: 79 - protein, 10 aa, synthetic construct
  REGION 1..10: note = Motif
AHGDAAHGCA

SEQ ID NO: 80 - protein, 10 aa, synthetic construct
  REGION 1..10: note = Motif
AHGDAADGHA

SEQ ID NO: 81 - protein, 10 aa, synthetic construct
  REGION 1..10: note = Motif
ACGHAAKGHA

SEQ ID NO: 82 - protein, 10 aa, synthetic construct
  REGION 1..10: note = Motif
ACGHAAHGKA

SEQ ID NO: 83 - protein, 10 aa, synthetic construct
  REGION 1..10: note = Motif
AHGCAAKGHA

SEQ ID NO: 84 - protein, 10 aa, synthetic construct
  REGION 1..10: note = Motif
AHGCAAHGKA

SEQ ID NO: 85 - protein, 10 aa, synthetic construct
  REGION 1..10: note = Motif
AKGHAAKGHA

SEQ ID NO: 86 - protein, 10 aa, synthetic construct
  REGION 1..10: note = Motif
AKGHAACGHA

SEQ ID NO: 87 - protein, 10 aa, synthetic construct
  REGION 1..10: note = Motif
AKGHAAHGCA

SEQ ID NO: 88 - protein, 10 aa, synthetic construct
  REGION 1..10: note = Motif
AKGHAAHGKA

SEQ ID NO: 89 - protein, 10 aa, synthetic construct
  REGION 1..10: note = Motif
AHGKAAHGKA

SEQ ID NO: 90 - protein, 10 aa, synthetic construct
  REGION 1..10: note = Motif
AHGKAACGHA

SEQ ID NO: 91 - protein, 10 aa, synthetic construct
  REGION 1..10: note = Motif
AHGKAAHGKA

SEQ ID NO: 92 - protein, 10 aa, synthetic construct
  REGION 1..10: note = Motif
AHGKAAKGHA

SEQ ID NO: 93 - protein, 10 aa, synthetic construct
  REGION 1..10: note = Motif
ACGHAAFGHA

SEQ ID NO: 94 - protein, 10 aa, synthetic construct
  REGION 1..10: note = Motif
ACGHAAHGFA

SEQ ID NO: 95 - protein, 10 aa, synthetic construct
  REGION 1..10: note = Motif
AHGCAAFGHA

SEQ ID NO: 96 - protein, 10 aa, synthetic construct
  REGION 1..10: note = Motif
AHGCAAHGFA

SEQ ID NO: 97 - protein, 10 aa, synthetic construct
  REGION 1..10: note = Motif
AFGHAAFGHA

SEQ ID NO: 98 - protein, 10 aa, synthetic construct
  REGION 1..10: note = Motif
AFGHAACGHA

SEQ ID NO: 99 - protein, 10 aa, synthetic construct
  REGION 1..10: note = Motif
AFGHAAHGCA

SEQ ID NO: 100 - protein, 10 aa, synthetic construct
  REGION 1..10: note = Motif
AFGHAAHGFA

SEQ ID NO: 101 - protein, 10 aa, synthetic construct
  REGION 1..10: note = Motif
AHGFAAHGFA

SEQ ID NO: 102 - protein, 10 aa, synthetic construct
  REGION 1..10: note = Motif
AHGFAACGHA

SEQ ID NO: 103 - protein, 10 aa, synthetic construct
  REGION 1..10: note = Motif
AHGFAAHGFA

SEQ ID NO: 104 - protein, 10 aa, synthetic construct
  REGION 1..10: note = Motif
AHGFAAFGHA

SEQ ID NO: 105 - DNA, 38 bp, synthetic construct
  misc_feature 1..38: note = Primer
  source 1..38: mol_type = other DNA
gctcctcgaggccaccatgggatggagctgtatcatcc

SEQ ID NO: 106 - DNA, 69 bp, synthetic construct
  misc_feature 1..69: note = Primer
  source 1..69: mol_type = other DNA
ccatgcggccgctcatttaggcatggccacaagcagcatggccacaggcacccggagacagggagaggc

SEQ ID NO: 107 - DNA, 38 bp, synthetic construct; identical to SEQ ID NO: 105
  misc_feature 1..38: note = Primer
  source 1..38: mol_type = other DNA

SEQ ID NO: 108 - DNA, 60 bp, synthetic construct
  misc_feature 1..60: note = Primer
  source 1..60: mol_type = other DNA
ccatgcggccgctcatttaggcatggccacaagcacctccaccacccggagacagggaga

SEQ ID NO: 109 - DNA, 38 bp, synthetic construct; identical to SEQ ID NO: 105
  misc_feature 1..38: note = Primer
  source 1..38: mol_type = other DNA

SEQ ID NO: 110 - DNA, 78 bp, synthetic construct
  misc_feature 1..78: note = Primer
  source 1..78: mol_type = other DNA
ccatgcggccgctcatttaggcatggccacaagcacctccaccagcatggccacaggcacccggagacagggagaggc

SEQ ID NO: 111 - DNA, 38 bp, synthetic construct; identical to SEQ ID NO: 105
  misc_feature 1..38: note = Primer
  source 1..38: mol_type = other DNA

SEQ ID NO: 112 - DNA, 63 bp, synthetic construct
  misc_feature 1..63: note = Primer
  source 1..63: mol_type = other DNA
cagattgcggccgctcattaggcatggccacaagcagcatggcctgaggcacccggagacagg

SEQ ID NO: 113 - DNA, 38 bp, synthetic construct; identical to SEQ ID NO: 105
  misc_feature 1..38: note = Primer
  source 1..38: mol_type = other DNA

SEQ ID NO: 114 - DNA, 63 bp, synthetic construct
  misc_feature 1..63: note = Primer
  source 1..63: mol_type = other DNA
cagattgcggccgctcattaggcatggcctgaagcagcatggccacaggcacccggagacagg

SEQ ID NO: 115 - protein, 448 aa, synthetic construct
  REGION 1..448: note = Heavy Chain of Fwt
EVQLVESGGGVVQPGRSLRLSCSASGFTFSGYGLSWVRQAPGKGLEWVAMISSGGSYTYYADSVKGRFAISRDNAKNTLFLQMDSLRPEDTGVYFCARHGDDPAWFAYWGQGTPVTVSSASTKGPSVFPLAPSSKSTSGGTAALGCLVKDYFPEPVTVSWNSGALTSGVHTFPAVLQSSGLYSLSSVVTVPSSSLGTQTYICNVNHKPSNTKVDKKVEPKSCDKTHTCPPCPAPELLGGPSVFLFPPKPKDTLMISRTPEVTCVVVDVSHEDPEVKFNWYVDGVEVHNAKTKPREEQYNSTYRVVSVLTVLHQDWLNGKEYKCKVSNKALPAPIEKTISKAKGQPREPQVYTLPPSRDELTKNQVSLTCLVKGFYPSDIAVEWESNGQPENNYKTTPPVLDSDGSFFLYSKLTVDKSRWQQGNVFSCSVMHEALHNHYTQKSLSLSPG

SEQ ID NO: 116 - protein, 217 aa, synthetic construct
  REGION 1..217: note = Light Chain of Fwt
DIQLTQSPSSLSASVGDRVTITCSVSSSISSNNLHWYQQKPGKAPKPWIYGTSNLASGVPSRFSGSGSGTDYTFTISSLQPEDIATYYCQQWSSYPYMYTFGQGTKVEIKRTVAAPSVFIFPPSDEQLKSGTASVVCLLNNFYPREAKVQWKVDNALQSGNSQESVTEQDSKDSTYSLSSTLTLSKADYEKHKVYACEVTHQGLSSPVTKSFNRGEC

SEQ ID NO: 117 - protein, 458 aa, synthetic construct
  REGION 1..458: note = FM2 Heavy Chain
EVQLVESGGGVVQPGRSLRLSCSASGFTFSGYGLSWVRQAPGKGLEWVAMISSGGSYTYYADSVKGRFAISRDNAKNTLFLQMDSLRPEDTGVYFCARHGDDPAWFAYWGQGTPVTVSSASTKGPSVFPLAPSSKSTSGGTAALGCLVKDYFPEPVTVSWNSGALTSGVHTFPAVLQSSGLYSLSSVVTVPSSSLGTQTYICNVNHKPSNTKVDKKVEPKSCDKTHTCPPCPAPELLGGPSVFLFPPKPKDTLMISRTPEVTCVVVDVSHEDPEVKFNWYVDGVEVHNAKTKPREEQYNSTYRVVSVLTVLHQDWLNGKEYKCKVSNKALPAPIEKTISKAKGQPREPQVYTLPPSRDELTKNQVSLTCLVKGFYPSDIAVEWESNGQPENNYKTTPPVLDSDGSFFLYSKLTVDKSRWQQGNVFSCSVMHEALHNHYTQKSLSLSPGACGHAACGHA

SEQ ID NO: 118 - protein, 458 aa, synthetic construct
  REGION 1..458: note = FM2a Heavy Chain
EVQLVESGGGVVQPGRSLRLSCSASGFTFSGYGLSWVRQAPGKGLEWVAMISSGGSYTYYADSVKGRFAISRDNAKNTLFLQMDSLRPEDTGVYFCARHGDDPAWFAYWGQGTPVTVSSASTKGPSVFPLAPSSKSTSGGTAALGCLVKDYFPEPVTVSWNSGALTSGVHTFPAVLQSSGLYSLSSVVTVPSSSLGTQTYICNVNHKPSNTKVDKKVEPKSCDKTHTCPPCPAPELLGGPSVFLFPPKPKDTLMISRTPEVTCVVVDVSHEDPEVKFNWYVDGVEVHNAKTKPREEQYNSTYRVVSVLTVLHQDWLNGKEYKCKVSNKALPAPIEKTISKAKGQPREPQVYTLPPSRDELTKNQVSLTCLVKGFYPSDIAVEWESNGQPENNYKTTPPVLDSDGSFFLYSKLTVDKSRWQQGNVFSCSVMHEALHNHYTQKSLSLSPGASGHAACGHA

SEQ ID NO: 119 - protein, 458 aa, synthetic construct
  REGION 1..458: note = FM2b Heavy Chain
EVQLVESGGGVVQPGRSLRLSCSASGFTFSGYGLSWVRQAPGKGLEWVAMISSGGSYTYYADSVKGRFAISRDNAKNTLFLQMDSLRPEDTGVYFCARHGDDPAWFAYWGQGTPVTVSSASTKGPSVFPLAPSSKSTSGGTAALGCLVKDYFPEPVTVSWNSGALTSGVHTFPAVLQSSGLYSLSSVVTVPSSSLGTQTYICNVNHKPSNTKVDKKVEPKSCDKTHTCPPCPAPELLGGPSVFLFPPKPKDTLMISRTPEVTCVVVDVSHEDPEVKFNWYVDGVEVHNAKTKPREEQYNSTYRVVSVLTVLHQDWLNGKEYKCKVSNKALPAPIEKTISKAKGQPREPQVYTLPPSRDELTKNQVSLTCLVKGFYPSDIAVEWESNGQPENNYKTTPPVLDSDGSFFLYSKLTVDKSRWQQGNVFSCSVMHEALHNHYTQKSLSLSPGACGHAASGHA

SEQ ID NO: 120 - protein, 456 aa, synthetic construct
  REGION 1..456: note = FM1 Heavy Chain
EVQLVESGGGVVQPGRSLRLSCSASGFTFSGYGLSWVRQAPGKGLEWVAMISSGGSYTYYADSVKGRFAISRDNAKNTLFLQMDSLRPEDTGVYFCARHGDDPAWFAYWGQGTPVTVSSASTKGPSVFPLAPSSKSTSGGTAALGCLVKDYFPEPVTVSWNSGALTSGVHTFPAVLQSSGLYSLSSVVTVPSSSLGTQTYICNVNHKPSNTKVDKKVEPKSCDKTHTCPPCPAPELLGGPSVFLFPPKPKDTLMISRTPEVTCVVVDVSHEDPEVKFNWYVDGVEVHNAKTKPREEQYNSTYRVVSVLTVLHQDWLNGKEYKCKVSNKALPAPIEKTISKAKGQPREPQVYTLPPSRDELTKNQVSLTCLVKGFYPSDIAVEWESNGQPENNYKTTPPVLDSDGSFFLYSKLTVDKSRWQQGNVFSCSVMHEALHNHYTQKSLSLSPGGGGACGHA

SEQ ID NO: 121 - protein, 461 aa, synthetic construct
  REGION 1..461: note = FM2L Heavy Chain
EVQLVESGGGVVQPGRSLRLSCSASGFTFSGYGLSWVRQAPGKGLEWVAMISSGGSYTYYADSVKGRFAISRDNAKNTLFLQMDSLRPEDTGVYFCARHGDDPAWFAYWGQGTPVTVSSASTKGPSVFPLAPSSKSTSGGTAALGCLVKDYFPEPVTVSWNSGALTSGVHTFPAVLQSSGLYSLSSVVTVPSSSLGTQTYICNVNHKPSNTKVDKKVEPKSCDKTHTCPPCPAPELLGGPSVFLFPPKPKDTLMISRTPEVTCVVVDVSHEDPEVKFNWYVDGVEVHNAKTKPREEQYNSTYRVVSVLTVLHQDWLNGKEYKCKVSNKALPAPIEKTISKAKGQPREPQVYTLPPSRDELTKNQVSLTCLVKGFYPSDIAVEWESNGQPENNYKTTPPVLDSDGSFFLYSKLTVDKSRWQQGNVFSCSVMHEALHNHYTQKSLSLSPGACGHAGGGACGHA

SEQ ID NO: 122 - protein, 131 aa, synthetic construct
  REGION 1..131: note = Fwt Hv
EVQLVESGGGVVQPGRSLRLSCSASGFTFSGYGLSWVRQAPGKGLEWVAMISSGGSYTYYADSVKGRFAISRDNAKNTLFLQMDSLRPEDTGVYFCARHGDDPAWFAYWGQGTPVTVSSASTKGPSVFPLA

SEQ ID NO: 123 - protein, 113 aa, synthetic construct
  REGION 1..113: note = Fwt Lv
DIQLTQSPSSLSASVGDRVTITCSVSSSISSNNLHWYQQKPGKAPKPWIYGTSNLASGVPSRFSGSGSGTDYTFTISSLQPEDIATYYCQQWSSYPYMYTFGQGTKVEIKRTV

SEQ ID NO: 124 - protein, 227 aa, synthetic construct
  REGION 1..227: note = Fwt Fab
EVQLVESGGGVVQPGRSLRLSCSASGFTFSGYGLSWVRQAPGKGLEWVAMISSGGSYTYYADSVKGRFAISRDNAKNTLFLQMDSLRPEDTGVYFCARHGDDPAWFAYWGQGTPVTVSSASTKGPSVFPLAPSSKSTSGGTAALGCLVKDYFPEPVTVSWNSGALTSGVHTFPAVLQSSGLYSLSSVVTVPSSSLGTQTYICNVNHKPSNTKVDKKVEPKSCDKTHT

SEQ ID NO: 125 - DNA, 1350 bp, synthetic construct
  misc_feature 1..1350: note = Fwt Heavy Chain
  source 1..1350: mol_type = other DNA
gaggtccaactggtggagagcggtggaggtgttgtgcaacctggccggtccctgcgcctgtcctgctccgcatctggcttcaccttcagcggctatgggttgtcttgggtgagacaggcacctggaaaaggtcttgagtgggttgcaatgattagtagtggtggtagttatacctactatgcagacagtgtgaagggtagatttgcaatatcgcgagacaacgccaagaacacattgttcctgcaaatggacagcctgagacccgaagacaccggggtctatttttgtgcaagacatggggacgatcccgcctggttcgcttattggggccaagggaccccggtcaccgtctcctcagcctccaccaagggcccatcggtcttccccctggcaccctcctccaagagcacctctgggggcacagcggccctgggctgcctggtcaaggactacttccccgaaccggtgacggtgtcgtggaactcaggcgccctgaccagcggcgtgcacaccttcccggctgtcctacagtcctcaggactctactccctcagcagcgtggtgaccgtgccctccagcagcttgggcacccagacctacatctgcaacgtgaatcacaagcccagcaacaccaaggtggacaagaaagttgagcccaaatcttgtgacaaaactcacacatgcccaccgtgcccagcacctgaactcctggggggaccgtcagtcttcctcttccccccaaaacccaaggacaccctcatgatctcccggacccctgaggtcacatgcgtggtggtggacgtgagccacgaagaccctgaggtcaagttcaactggtacgtggacggcgtggaggtgcataatgccaagacaaagccgcgggaggagcagtacaacagcacgtaccgtgtggtcagcgtcctcaccgtcctgcaccaggactggctgaatggcaaggagtacaagtgcaaggtctccaacaaagccctcccagcccccatcgagaaaaccatctccaaagccaaagggcagccccgagaaccacaggtgtacaccctgcccccatcccgggatgagctgaccaagaaccaggtcagcctgacctgcctggtcaaaggcttctatcccagcgacatcgccgtggagtgggagagcaatgggcagccggagaacaactacaagaccacgcctcccgtgctggactccgacggctccttcttcctctacagcaagctcaccgtggacaagagcaggtggcagcaggggaacgtcttctcatgctccgtgatgcatgaggctctgcacaaccactacacgcagaagagcctctccctgtctcccgggaaatga

SEQ ID NO: 126 - DNA, 654 bp, synthetic construct
  misc_feature 1..654: note = Fwt Light Chain
  source 1..654: mol_type = other DNA
gacatccagctgacccagagcccaagcagcctgagcgccagcgtgggtgacagagtgaccatcacctgtagtgtcagctcaagtataagttccaacaacttgcactggtaccagcagaagccaggtaaggctccaaagccatggatctacggcacatccaacctggcttctggtgtgccaagcagattcagcggtagcggtagcggtaccgactacaccttcaccatcagcagcctccagccagaggacatcgccacctactactgccaacagtggagtagttacccgtacatgtacacgttcggccaagggaccaaggtggaaatcaaacgaactgtggctgcaccatctgtcttcatcttcccgccatctgatgagcagttgaaatctggaactgcctctgttgtgtgcctgctgaataacttctatcccagagaggccaaagtacagtggaaggtggataacgccctccaatcgggtaactcccaggagagtgtcacagagcaggacagcaaggacagcacctacagcctcagcagcaccctgacgctgagcaaagcagactacgagaaacacaaagtctacgcctgcgaagtcacccatcagggcctgagctcgcccgtcacaaagagcttcaacaggggagagtgttaa

SEQ ID NO: 127 - protein, 451 aa, synthetic construct
  REGION 1..451: note = Trastuzumab Heavy chain
EVQLVESGGGLVQPGGSLRLSCAASGFNIKDTYIHWVRQAPGKGLEWVARIYPTNGYTRYADSVKGRFTISADTSKNTAYLQMNSLRAEDTAVYYCSRWGGDGFYAMDYWGQGTLVTVSSASTKGPSVFPLAPSSKSTSGGTAALGCLVKDYFPEPVTVSWNSGALTSGVHTFPAVLQSSGLYSLSSVVTVPSSSLGTQTYICNVNHKPSNTKVDKKVEPPKSCDKTHTCPPCPAPELLGGPSVFLFPPKPKDTLMISRTPEVTCVVVDVSHEDPEVKFNWYVDGVEVHNAKTKPREEQYNSTYRVVSVLTVLHQDWLNGKEYKCKVSNKALPAPIEKTISKAKGQPREPQVYTLPPSRDELTKNQVSLTCLVKGFYPSDIAVEWESNGQPENNYKTTPPVLDSDGSFFLYSKLTVDKSRWQQGNVFSCSVMHEALHNHYTQKSLSLSPGK

SEQ ID NO: 128 - protein, 214 aa, synthetic construct
  REGION 1..214: note = Trastuzumab Light chain
DIQMTQSPSSLSASVGDRVTITCRASQDVNTAVAWYQQKPGKAPKLLIYSASFLYSGVPSRFSGSRSGTDFTLTISSLQPEDFATYYCQQHYTTPPTFGQGTKVEIKRTVAAPSVFIFPPSDEQLKSGTASVVCLLNNFYPREAKVQWKVDNALQSGNSQESVTEQDSKDSTYSLSSTLTLSKADYEKHKVYACEVTHQGLSSPVTKSFNRGEC